European Patent Application EP 4 265 727 A1, published October 25, 2023. Title: Mutant Glucose Dehydrogenase. Applicant: Amano Enzyme Inc. Tokyo University of Agriculture and Technology University of North Carolina at Chapel Hill. The sequence listing filed with the application follows.

SEQUENCE LISTING (22 sequences)

SEQ ID NO: 1 - protein, 605 aa, Artificial Sequence
  double mutant (D446H, V582P) of glucose oxidase derived from Aspergillus niger
MSTLLVSSLVVSLAAALPHYIRSNGIEASLLTDPKEVAGRTVDYIIAGGGLTGLTTAARLTENPDITVLVIESGSYESDRGPIIEDLNAYGDIFGSSVDHAYETVELATNNQTALIRSGNGLGGSTLVNGGTWTRPHKAQVDSWETVFGNEGWNWDSVAAYSLQAERARAPNAKQIAAGHYFNASCHGINGTVHAGPRDTGDDYSPIVKALMSAVEDRGVPTKKDLGCGDPHGVSMFPNTLHEDQVRSDAAREWLLPNYQRPNLQVLTGRYVGKVLLSQNATTPRAVGVEFGTHKGNTHNVYAKHEVLLAAGSAVSPTILEYSGIGMKSILEPLGIDTVVDLPVGLNLQDQTTSTVRSRITSAGAGQGQAAWFATFNETFGDYAEKAHELLNTKLEQWAEEAVARGGFHNTTALLIQYENYRDWIVKDNVAYSELFLDTAGVASFHVWDLLPFTRGYVHILDKDPYLRHFAYDPQYFLNELDLLGQAAATQLARNISNSGAMQTYFAGETIPGDNLAYDADLSAWVEYIPYNFRPNYHGVGTCSMMPKEMGGVVDNAARVYGVQGLRVIDGSIPPTQMSSHPMTVFYAMALKVADAILADYASMQ

SEQ ID NO: 2 - DNA, 1818 bp, Artificial Sequence
  DNA coding double mutant (D446H, V582P) of glucose oxidase derived from Aspergillus niger
atgtctactctccttgtgagctcgcttgtggtctccctcgctgcggccctcccacactacatcaggagcaatggcatcgaagccagcctcctgactgaccccaaggaggttgccggccgcactgtcgactacatcatcgctggtggaggtctgactggactcaccactgctgcccgtctgacggagaaccccgatatcactgtgcttgtcatcgaaagtggctcctacgagtctgacagaggtcctatcattgaggacctgaacgcttacggtgacatttttggcagcagtgtggaccacgcctacgagactgtcgagctcgccaccaacaatcagactgcgctgatccgctccggaaatggtctcggtggctctaccctcgtcaacggtggcacctggactcgcccccacaaggcacaagttgactcatgggagaccgtcttcggaaatgagggctggaactgggacagcgtggccgcctactccctccaggctgagcgtgctcgcgcaccaaatgccaaacagattgctgctggccactactttaatgcatcctgccatggtatcaatggtactgtccacgccggaccccgcgataccggtgatgactactcccccatcgtcaaggctctcatgagcgctgtcgaagacaggggcgttcccaccaagaaggacttgggatgcggtgacccccatggtgtgtccatgttccccaacaccttgcacgaagaccaagtgcgctctgatgccgctcgtgaatggctcctccccaactaccagcgtcccaacctgcaagtcctcactggacggtatgttggaaaggtcctgctcagccagaacgctaccacacctcgtgccgttggcgtggaattcggcacccacaagggcaacacccacaacgtctacgctaagcacgaggtcctcctggccgctggatccgctgtctctcccaccatcctcgaatattccggtatcggaatgaagtccattctagagcctcttggaattgacaccgtcgttgacctgcccgttggtctcaaccttcaggaccagaccacctctaccgtccgctcacgcattacctccgccggtgccggacagggacaggccgcttggttcgctaccttcaacgagacctttggcgactacgccgaaaaggctcacgagctgctcaacaccaagctggagcagtgggccgaagaggccgtcgcccgtggcggattccacaacaccaccgctttgctcatccagtacgagaactaccgcgactggatcgtcaaggacaatgtcgcatactcggaactcttcctcgacacggccggagtggccagtttccatgtgtgggatcttctgcccttcactagaggatacgtacacatcctcgacaaggacccctacctccgccatttcgcatacgaccctcagtactttctcaacgagcttgacctgctcggccaggctgccgccactcagctggcccgcaacatctccaactccggtgccatgcaaacttatttcgctggagagactattcccggtgacaacctcgcgtatgatgccgacttgagcgcctgggttgagtatatcccgtacaacttccgccctaactaccatggtgtgggtacttgctccatgatgccgaaggagatgggcggtgttgtcgacaatgctgcccgtgtgtatggtgtgcagggactgcgagtcatcgatggttctattccccctacgcaaatgtcgtcccatcctatgacggtcttttatgccatggccttgaaggttgcggatgccatcttggcggattatgcttccatgcagtga

SEQ ID NO: 3 - DNA, 1818 bp, Artificial Sequence
  DNA coding mutant (M578V) of double mutant shown in SEQ No.1
atgtctactctccttgtgagctcgcttgtggtctccctcgctgcggccctcccacactacatcaggagcaatggcatcgaagccagcctcctgactgaccccaaggaggttgccggccgcactgtcgactacatcatcgctggtggaggtctgactggactcaccactgctgcccgtctgacggagaaccccgatatcactgtgcttgtcatcgaaagtggctcctacgagtctgacagaggtcctatcattgaggacctgaacgcttacggtgacatttttggcagcagtgtggaccacgcctacgagactgtcgagctcgccaccaacaatcagactgcgctgatccgctccggaaatggtctcggtggctctaccctcgtcaacggtggcacctggactcgcccccacaaggcacaagttgactcatgggagaccgtcttcggaaatgagggctggaactgggacagcgtggccgcctactccctccaggctgagcgtgctcgcgcaccaaatgccaaacagattgctgctggccactactttaatgcatcctgccatggtatcaatggtactgtccacgccggaccccgcgataccggtgatgactactcccccatcgtcaaggctctcatgagcgctgtcgaagacaggggcgttcccaccaagaaggacttgggatgcggtgacccccatggtgtgtccatgttccccaacaccttgcacgaagaccaagtgcgctctgatgccgctcgtgaatggctcctccccaactaccagcgtcccaacctgcaagtcctcactggacggtatgttggaaaggtcctgctcagccagaacgctaccacacctcgtgccgttggcgtggaattcggcacccacaagggcaacacccacaacgtctacgctaagcacgaggtcctcctggccgctggatccgctgtctctcccaccatcctcgaatattccggtatcggaatgaagtccattctagagcctcttggaattgacaccgtcgttgacctgcccgttggtctcaaccttcaggaccagaccacctctaccgtccgctcacgcattacctccgccggtgccggacagggacaggccgcttggttcgctaccttcaacgagacctttggcgactacgccgaaaaggctcacgagctgctcaacaccaagctggagcagtgggccgaagaggccgtcgcccgtggcggattccacaacaccaccgctttgctcatccagtacgagaactaccgcgactggatcgtcaaggacaatgtcgcatactcggaactcttcctcgacacggccggagtggccagtttccatgtgtgggatcttctgcccttcactagaggatacgtacacatcctcgacaaggacccctacctccgccatttcgcatacgaccctcagtactttctcaacgagcttgacctgctcggccaggctgccgccactcagctggcccgcaacatctccaactccggtgccatgcaaacttatttcgctggagagactattcccggtgacaacctcgcgtatgatgccgacttgagcgcctgggttgagtatatcccgtacaacttccgccctaactaccatggtgtgggtacttgctccatgatgccgaaggagatgggcggtgttgtcgacaatgctgcccgtgtgtatggtgtgcagggactgcgagtcatcgatggttctattccccctacgcaagtgtcgtcccatcctatgacggtcttttatgccatggccttgaaggttgcggatgccatcttggcggattatgcttccatgcagtga

SEQ ID NO: 4 - DNA, 1818 bp, Artificial Sequence
  DNA coding mutant (M578F) of double mutant shown in SEQ No.1
atgtctactctccttgtgagctcgcttgtggtctccctcgctgcggccctcccacactacatcaggagcaatggcatcgaagccagcctcctgactgaccccaaggaggttgccggccgcactgtcgactacatcatcgctggtggaggtctgactggactcaccactgctgcccgtctgacggagaaccccgatatcactgtgcttgtcatcgaaagtggctcctacgagtctgacagaggtcctatcattgaggacctgaacgcttacggtgacatttttggcagcagtgtggaccacgcctacgagactgtcgagctcgccaccaacaatcagactgcgctgatccgctccggaaatggtctcggtggctctaccctcgtcaacggtggcacctggactcgcccccacaaggcacaagttgactcatgggagaccgtcttcggaaatgagggctggaactgggacagcgtggccgcctactccctccaggctgagcgtgctcgcgcaccaaatgccaaacagattgctgctggccactactttaatgcatcctgccatggtatcaatggtactgtccacgccggaccccgcgataccggtgatgactactcccccatcgtcaaggctctcatgagcgctgtcgaagacaggggcgttcccaccaagaaggacttgggatgcggtgacccccatggtgtgtccatgttccccaacaccttgcacgaagaccaagtgcgctctgatgccgctcgtgaatggctcctccccaactaccagcgtcccaacctgcaagtcctcactggacggtatgttggaaaggtcctgctcagccagaacgctaccacacctcgtgccgttggcgtggaattcggcacccacaagggcaacacccacaacgtctacgctaagcacgaggtcctcctggccgctggatccgctgtctctcccaccatcctcgaatattccggtatcggaatgaagtccattctagagcctcttggaattgacaccgtcgttgacctgcccgttggtctcaaccttcaggaccagaccacctctaccgtccgctcacgcattacctccgccggtgccggacagggacaggccgcttggttcgctaccttcaacgagacctttggcgactacgccgaaaaggctcacgagctgctcaacaccaagctggagcagtgggccgaagaggccgtcgcccgtggcggattccacaacaccaccgctttgctcatccagtacgagaactaccgcgactggatcgtcaaggacaatgtcgcatactcggaactcttcctcgacacggccggagtggccagtttccatgtgtgggatcttctgcccttcactagaggatacgtacacatcctcgacaaggacccctacctccgccatttcgcatacgaccctcagtactttctcaacgagcttgacctgctcggccaggctgccgccactcagctggcccgcaacatctccaactccggtgccatgcaaacttatttcgctggagagactattcccggtgacaacctcgcgtatgatgccgacttgagcgcctgggttgagtatatcccgtacaacttccgccctaactaccatggtgtgggtacttgctccatgatgccgaaggagatgggcggtgttgtcgacaatgctgcccgtgtgtatggtgtgcagggactgcgagtcatcgatggttctattccccctacgcaattctcgtcccatcctatgacggtcttttatgccatggccttgaaggttgcggatgccatcttggcggattatgcttccatgcagtga

SEQ ID NO: 5 - DNA, 27 bp, Artificial Sequence
  primer for obtaining M578A mutatnt
acgcaagcctcgtcccatcctatgacg

SEQ ID NO: 6 - DNA, 27 bp, Artificial Sequence
  primer for obtaining M578A mutatnt
ggacgaggcttgcgtagggggaataga

SEQ ID NO: 7 - DNA, 27 bp, Artificial Sequence
  primer for obtaining M578N mutatnt
acgcaaaactcgtcccatcctatgacg

SEQ ID NO: 8 - DNA, 27 bp, Artificial Sequence
  primer for obtaining M578N mutatnt
ggacgagttttgcgtagggggaataga

SEQ ID NO: 9 - DNA, 27 bp, Artificial Sequence
  primer for obtaining M578V mutatnt
acgcaagtgtcgtcccatcctatgacg

SEQ ID NO: 10 - DNA, 27 bp, Artificial Sequence
  primer for obtaining M578V mutatnt
ggacgacacttgcgtagggggaataga

SEQ ID NO: 11 - DNA, 25 bp, Artificial Sequence
  primer for obtaining M578L mutatnt
tacgcaactgtcgtcccatcctatg

SEQ ID NO: 12 - DNA, 25 bp, Artificial Sequence
  primer for obtaining M578L mutatnt
gacgacagttgcgtagggggaatag

SEQ ID NO: 13 - DNA, 27 bp, Artificial Sequence
  primer for obtaining M578K mutatnt
acgcaaaagtcgtcccatcctatgacg

SEQ ID NO: 14 - DNA, 27 bp, Artificial Sequence
  primer for obtaining M578K mutatnt
ggacgacttttgcgtagggggaataga

SEQ ID NO: 15 - DNA, 27 bp, Artificial Sequence
  primer for obtaining M578D mutatnt
acgcaagattcgtcccatcctatgacg

SEQ ID NO: 16 - DNA, 27 bp, Artificial Sequence
  primer for obtaining M578D mutatnt
ggacgaatcttgcgtagggggaataga

SEQ ID NO: 17 - DNA, 27 bp, Artificial Sequence
  primer for obtaining M578F mutatnt
acgcaattctcgtcccatcctatgacg

SEQ ID NO: 18 - DNA, 27 bp, Artificial Sequence
  primer for obtaining M578F mutatnt
ggacgagaattgcgtagggggaataga

SEQ ID NO: 19 - DNA, 27 bp, Artificial Sequence
  primer for obtaining M578W mutatnt
acgcaatggtcgtcccatcctatgacg

SEQ ID NO: 20 - DNA, 27 bp, Artificial Sequence
  primer for obtaining M578W mutatnt
ggacgaccattgcgtagggggaataga

SEQ ID NO: 21 - DNA, 27 bp, Artificial Sequence
  primer for obtaining M578Y mutatnt
acgcaatactcgtcccatcctatgacg

SEQ ID NO: 22 - DNA, 27 bp, Artificial Sequence
  primer for obtaining M578Y mutatnt
ggacgagtattgcgtagggggaataga